European Patent Application EP 4 628 580 A1, published October 8, 2025. Title: ＤＮＡを二本鎖切断するヌクレアーゼドメイン. Applicant: Hiroshima University. Application JP. The sequence listing filed with the application follows.

SEQUENCE LISTING (97 sequences)

SEQ ID NO: 1 - DNA, 21 bp, synthetic construct
  misc_feature 1..21: note = FokI_FW
  source 1..21: mol_type = other DNA
cacagagtggccctgaagcag

SEQ ID NO: 2 - DNA, 21 bp, synthetic construct
  misc_feature 1..21: note = FokI_RV
  source 1..21: mol_type = other DNA
gccactgtgctggattaaaag

SEQ ID NO: 3 - DNA, 43 bp, synthetic construct
  misc_feature 1..43: note = TALE63-RinfFokI
  source 1..43: mol_type = other DNA
cagggccactctgtgtgatgtcctctcggggatccttctgttg

SEQ ID NO: 4 - DNA, 42 bp, synthetic construct
  misc_feature 1..42: note = Vector-FinfFokI
  source 1..42: mol_type = other DNA
atccagcacagtggcgaattctgcagatatccagcacagtgg

SEQ ID NO: 5 - DNA, 45 bp, synthetic construct
  misc_feature 1..45: note = ND1F_inf63-2
  source 1..45: mol_type = other DNA
cgagtggcaggttcccttgttaagggcgaaatggagaaaaagaag

SEQ ID NO: 6 - DNA, 48 bp, synthetic construct
  misc_feature 1..48: note = ND1R_inf63
  source 1..48: mol_type = other DNA
atatctgcagaattcttagaagatgatctcgtcattgttgaacttatc

SEQ ID NO: 7 - DNA, 42 bp, synthetic construct
  misc_feature 1..42: note = ND2F_inf63
  source 1..42: mol_type = other DNA
cgagtggcaggttccattgttaagagcagcattgagatgagc

SEQ ID NO: 8 - DNA, 46 bp, synthetic construct
  misc_feature 1..46: note = ND2R_inf63
  source 1..46: mol_type = other DNA
atatctgcagaattcttagaactgaatctccttattcaggaaagag

SEQ ID NO: 9 - DNA, 48 bp, synthetic construct
  misc_feature 1..48: note = ND1monoR_inf63
  source 1..48: mol_type = other DNA
atatctgcagaattcttaaaagataatctcatcgttgttgaatttatc

SEQ ID NO: 10 - DNA, 49 bp, synthetic construct
  misc_feature 1..49: note = ND2monoR_inf63
  source 1..49: mol_type = other DNA
atatctgcagaattcttagaactggatctctttgttcagaaacgaattc

SEQ ID NO: 11 - DNA, 26 bp, synthetic construct
  misc_feature 1..26: note = TALE_63_R
  source 1..26: mol_type = other DNA
ggaacctgccactcgatgtgatgtcc

SEQ ID NO: 12 - DNA, 27 bp, synthetic construct
  misc_feature 1..27: note = TALEvector_F
  source 1..27: mol_type = other DNA
gaattctgcagatatccagcacagtgg

SEQ ID NO: 13 - DNA, 24 bp, synthetic construct
  misc_feature 1..24: note = TALE_47_R
  source 1..24: mol_type = other DNA
ggatctgatcaattccggcgcgtg

SEQ ID NO: 14 - DNA, 39 bp, synthetic construct
  misc_feature 1..39: note = EGFP_F+bam
  source 1..39: mol_type = other DNA
taccgagctcggatcatggtgagcaagggcgaggagctg

SEQ ID NO: 15 - DNA, 21 bp, synthetic construct
  misc_feature 1..21: note = EGFP_600R
  source 1..21: mol_type = other DNA
gtggttgtcgggcagcagcac

SEQ ID NO: 16 - DNA, 36 bp, synthetic construct
  misc_feature 1..36: note = EGFP_600R+linker
  source 1..36: mol_type = other DNA
gctagcggatcctcagtggttgtcgggcagcagcac

SEQ ID NO: 17 - DNA, 24 bp, synthetic construct
  misc_feature 1..24: note = EGFP_120F
  source 1..24: mol_type = other DNA
ggcaagctgaccctgaagttcatc

SEQ ID NO: 18 - DNA, 40 bp, synthetic construct
  misc_feature 1..40: note = EGFP_R+rv
  source 1..40: mol_type = other DNA
gccactgtgctggatttacttgtacagctcgtccatgccg

SEQ ID NO: 19 - DNA, 63 bp, synthetic construct
  misc_feature 1..63: note = linker+EGFP_120F
  source 1..63: mol_type = other DNA
tgaggatccgctagcctgcaggtcgacgaattcgatatcggcaagctgaccctgaagttcatc

SEQ ID NO: 20 - DNA, 27 bp, synthetic construct
  misc_feature 1..27: note = TALE-CR
  source 1..27: mol_type = other DNA
gagacgaccggtggaaagcgggcagtg

SEQ ID NO: 21 - DNA, 24 bp, synthetic construct
  misc_feature 1..24: note = Amp_R
  source 1..24: mol_type = other DNA
cactcatggttatggcagcactgc

SEQ ID NO: 22 - DNA, 30 bp, synthetic construct
  misc_feature 1..30: note = ND1-N_F
  source 1..30: mol_type = other DNA
cttgttaagggcgaaatggagaaaaagaag

SEQ ID NO: 23 - DNA, 29 bp, synthetic construct
  misc_feature 1..29: note = Amp_F
  source 1..29: mol_type = other DNA
ccataaccatgagtgataacactgcggcc

SEQ ID NO: 24 - DNA, 29 bp, synthetic construct
  misc_feature 1..29: note = WT-CF
  source 1..29: mol_type = other DNA
tccaccggtcgtctccacccctgagcagg

SEQ ID NO: 25 - DNA, 42 bp, synthetic construct
  misc_feature 1..42: note = WT-63R_infND1
  source 1..42: mol_type = other DNA
ttcgcccttaacaagtgccactcgatgtgatgtcctctcggg

SEQ ID NO: 26 - DNA, 42 bp, synthetic construct
  misc_feature 1..42: note = WT-75R_infND1
  source 1..42: mol_type = other DNA
ttcgcccttaacaaggaagaatccgagcacgcggaccacttg

SEQ ID NO: 27 - DNA, 41 bp, synthetic construct
  misc_feature 1..41: note = WT-90R_infND1
  source 1..41: mol_type = other DNA
ttcgcccttaacaagagtcatggcgtcatcgaacgcttgtg

SEQ ID NO: 28 - DNA, 44 bp, synthetic construct
  misc_feature 1..44: note = WT-105R_infND1
  source 1..44: mol_type = other DNA
ttcgcccttaacaagtctacgaaagagctgcagcagtccgtgtc

SEQ ID NO: 29 - DNA, 43 bp, synthetic construct
  misc_feature 1..43: note = WT-120_infND1
  source 1..43: mol_type = other DNA
ttcgcccttaacaaggggaggcagtgtgcccgagcgggcctcc

SEQ ID NO: 30 - DNA, 43 bp, synthetic construct
  misc_feature 1..43: note = WT-135R_infND1
  source 1..43: mol_type = other DNA
ttcgcccttaacaagtttcataccgctcgcttggagaatcctg

SEQ ID NO: 31 - DNA, 41 bp, synthetic construct
  misc_feature 1..41: note = WT-150R_infND1
  source 1..41: mol_type = other DNA
ttcgcccttaacaagcgcctggtcaggtgtctgagttgacg

SEQ ID NO: 32 - DNA, 42 bp, synthetic construct
  misc_feature 1..42: note = WT-165R_infND1
  source 1..42: mol_type = other DNA
ttcgcccttaacaagcgcgtccaaatccctctccagcgagtc

SEQ ID NO: 33 - DNA, 42 bp, synthetic construct
  misc_feature 1..42: note = WT-180R_infND1
  source 1..42: mol_type = other DNA
ttcgcccttaacaaggctggctgacgcgcgagtttggtcccc

SEQ ID NO: 34 - DNA, 43 bp, synthetic construct
  misc_feature 1..43: note = TALE-0_R_infND1
  source 1..43: mol_type = other DNA
ttcgcccttaacaagctccagtgcgggtctgcccccgttgttg

SEQ ID NO: 35 - DNA, 43 bp, synthetic construct
  misc_feature 1..43: note = TALE-12_R_infND1
  source 1..43: mol_type = other DNA
ttcgcccttaacaagcgcggggtccggcctcgaaagctgggcc

SEQ ID NO: 36 - DNA, 41 bp, synthetic construct
  misc_feature 1..41: note = TALE-24_R_infND1
  source 1..41: mol_type = other DNA
ttcgcccttaacaagcgctacaagatgatcattagtgagtg

SEQ ID NO: 37 - DNA, 42 bp, synthetic construct
  misc_feature 1..42: note = TALE-36_R_infND1
  source 1..42: mol_type = other DNA
ttcgcccttaacaagcactgcatccatggcaggacgtccgcc

SEQ ID NO: 38 - DNA, 41 bp, synthetic construct
  misc_feature 1..41: note = GSSx4+5'ad._F
  source 1..41: mol_type = other DNA
ccgggtggggtctagtggctccagcggatcaagtggcagct

SEQ ID NO: 39 - DNA, 41 bp, synthetic construct
  misc_feature 1..41: note = GSSx4+5'ad._R
  source 1..41: mol_type = other DNA
ccggagctgccacttgatccgctggagccactagaccccac

SEQ ID NO: 40 - DNA, 41 bp, synthetic construct
  misc_feature 1..41: note = SAGGx3+5'ad._F
  source 1..41: mol_type = other DNA
ccgggtgtctgctggcgggtccgccgggggcagtgctggcg

SEQ ID NO: 41 - DNA, 41 bp, synthetic construct
  misc_feature 1..41: note = SAGGx3+5'ad._R
  source 1..41: mol_type = other DNA
gatccgccagcactgcccccggcggacccgccagcagacac

SEQ ID NO: 42 - DNA, 50 bp, synthetic construct
  misc_feature 1..50: note = GGGGSx3+5'ad._F
  source 1..50: mol_type = other DNA
ccgggtggggggcggagggtctggcggagggggctctggagggggcggat

SEQ ID NO: 43 - DNA, 50 bp, synthetic construct
  misc_feature 1..50: note = GGGGSx3+5'ad._R
  source 1..50: mol_type = other DNA
ccggatccgccccctccagagccccctccgccagaccctccgccccccac

SEQ ID NO: 44 - DNA, 36 bp, synthetic construct
  misc_feature 1..36: note = GSSx4_F
  source 1..36: mol_type = other DNA
ccgggtctagtggctccagcggatcaagtggcagct

SEQ ID NO: 45 - DNA, 36 bp, synthetic construct
  misc_feature 1..36: note = GSSx4_R
  source 1..36: mol_type = other DNA
ccggagctgccacttgatccgctggagccactagac

SEQ ID NO: 46 - DNA, 63 bp, synthetic construct
  misc_feature 1..63: note = GSSx7_F
  source 1..63: mol_type = other DNA
ccgggtctagtggctccagcggatcaagtgggagttctggcagctcaggatctagtggcagct

SEQ ID NO: 47 - DNA, 63 bp, synthetic construct
  misc_feature 1..63: note = GSSx7_R
  source 1..63: mol_type = other DNA
ccggagctgccactagatcctgagctgccagaactcccacttgatccgctggagccactagac

SEQ ID NO: 48 - DNA, 36 bp, synthetic construct
  misc_feature 1..36: note = SAGGx3_F
  source 1..36: mol_type = other DNA
gatctgctggcgggtccgccgggggcagtgctggcg

SEQ ID NO: 49 - DNA, 36 bp, synthetic construct
  misc_feature 1..36: note = SAGGx3_R
  source 1..36: mol_type = other DNA
gatccgccagcactgcccccggcggacccgccagca

SEQ ID NO: 50 - DNA, 48 bp, synthetic construct
  misc_feature 1..48: note = SAGGx4_F
  source 1..48: mol_type = other DNA
gatctgctggcgggtccgccgggggctcagcaggagggagtgctggcg

SEQ ID NO: 51 - DNA, 48 bp, synthetic construct
  misc_feature 1..48: note = SAGGx4_R
  source 1..48: mol_type = other DNA
gatccgccagcactccctcctgctgagcccccggcggacccgccagca

SEQ ID NO: 52 - DNA, 45 bp, synthetic construct
  misc_feature 1..45: note = GGGGSx3_F
  source 1..45: mol_type = other DNA
ccgggggcggagggtctggcggagggggctctggagggggcggat

SEQ ID NO: 53 - DNA, 45 bp, synthetic construct
  misc_feature 1..45: note = GGGGSx3_R
  source 1..45: mol_type = other DNA
ccggatccgccccctccagagccccctccgccagaccctccgccc

SEQ ID NO: 54 - DNA, 60 bp, synthetic construct
  misc_feature 1..60: note = GGGGSx4_F
  source 1..60: mol_type = other DNA
ccgggggcggagggtctggcggagggggctctggagggggcggatcagggggcggagggt

SEQ ID NO: 55 - DNA, 60 bp, synthetic construct
  misc_feature 1..60: note = GGGGSx4_R
  source 1..60: mol_type = other DNA
ccggaccctccgccccctgatccgccccctccagagccccctccgccagaccctccgccc

SEQ ID NO: 56 - DNA, 33 bp, synthetic construct
  misc_feature 1..33: note = bamND1_F
  source 1..33: mol_type = other DNA
ggatccatgaccgcggtcctcgtgaaaggggag

SEQ ID NO: 57 - DNA, 42 bp, synthetic construct
  misc_feature 1..42: note = 95aa_R_inf_bamND1
  source 1..42: mol_type = other DNA
cgcggtcatggatccgctagatccgcttccagatccgctgcc

SEQ ID NO: 58 - DNA, 33 bp, synthetic construct
  misc_feature 1..33: note = mroND1_F
  source 1..33: mol_type = other DNA
tccggaatgaccgcggtcctcgtgaaaggggag

SEQ ID NO: 59 - DNA, 42 bp, synthetic construct
  misc_feature 1..42: note = 95aa_R_inf_mroND1
  source 1..42: mol_type = other DNA
cgcggtcattccggagctagatccgcttccagatccgctgcc

SEQ ID NO: 60 - DNA, 1461 bp, synthetic construct
  misc_feature 1..1461: note = FokI-95-FokI
  source 1..1461: mol_type = other DNA
  CDS 1..1461
cagctggtgaagtctgagctggaggagaagaagagcgagctgcggcacaagctgaagtacgtgccacacgagtatatcgagctgatcgagatcgcccggaactccacccaggacagaatcctggagatgaaagtgatggagttctttatgaaggtgtacggatataggggcaagcacctgggaggctccagaaagcctgatggcgccatctacaccgtgggctctccaatcgactatggcgtgatcgtggatacaaaggcctactccggcggctataatctgcccatcggccaggccgatgagatgcagaggtacgtggaggagaaccagacccgcaataagcacatcaaccccaatgagtggtggaaggtgtatcctagctccgtgacagagttcaagtttctgttcgtgtctggccacttcaagggcaactacaaggcccagctgaccagactgaatcacatcacaaactgtaatggagccgtgctgagcgtggaggagctgctgatcggcggcgagatgatcaaggcaggcaccctgacactggaggaggtgcggagaaagttcaacaatggcgagatcaactttggaagcggatccggatctggaagcatcaccaggaccacaaaccctcgcaatgtggtgccaaagatctacatgtccgccggctctatccctctgaccacacacatcacaaacagcatccagccaaccctgtggacaatcggatccatcaatggagtggcaccactggccaagtctatcaagctgggcatccctgtgaccggcagcgcctacacagaccagaccacagccatggtgcggaagaaggtgagcgtgttcatgggcagcggatctggaagcggatctagccagctggtgaagtccgaactggaagagaagaagtctgagctgcgccataagctgaagtatgtgcctcatgaatacattgaactgattgagatcgccaggaacagcacccaggaccgcatcctggaaatgaaagtgatggagttctttatgaaagtctatggctacagaggcaagcacctgggcggcagcagaaagccagacggagctatctacactgtgggctcccccattgattacggcgtgatcgtcgatacaaaggcctacagtggaggatacaatctgcctattggacaggctgatgagatgcagaggtatgtggaggaaaatcagactagaaataagcacatcaacccaaacgaatggtggaaggtgtacccctcctctgtgacagagtttaagttcctgttcgtgagcggacacttcaagggaaactataaggcccagctgacccggctgaatcatattacaaactgcaatggcgccgtgctgtctgtcgaagaactgctgattggaggagagatgatcaaggccggcaccctgacactggaagaggtgaggcgcaagttcaacaacggagagatcaacttt

SEQ ID NO: 61 - protein, 487 aa, synthetic construct
  REGION 1..487: note = Synthetic Construct
QLVKSELEEKKSELRHKLKYVPHEYIELIEIARNSTQDRILEMKVMEFFMKVYGYRGKHLGGSRKPDGAIYTVGSPIDYGVIVDTKAYSGGYNLPIGQADEMQRYVEENQTRNKHINPNEWWKVYPSSVTEFKFLFVSGHFKGNYKAQLTRLNHITNCNGAVLSVEELLIGGEMIKAGTLTLEEVRRKFNNGEINFGSGSGSGSITRTTNPRNVVPKIYMSAGSIPLTTHITNSIQPTLWTIGSINGVAPLAKSIKLGIPVTGSAYTDQTTAMVRKKVSVFMGSGSGSGSSQLVKSELEEKKSELRHKLKYVPHEYIELIEIARNSTQDRILEMKVMEFFMKVYGYRGKHLGGSRKPDGAIYTVGSPIDYGVIVDTKAYSGGYNLPIGQADEMQRYVEENQTRNKHINPNEWWKVYPSSVTEFKFLFVSGHFKGNYKAQLTRLNHITNCNGAVLSVEELLIGGEMIKAGTLTLEEVRRKFNNGEINF

SEQ ID NO: 62 - DNA, 1356 bp, synthetic construct
  misc_feature 1..1356: note = FokI-60-FokI
  source 1..1356: mol_type = other DNA
  CDS 1..1356
cagctggtgaagtccgagctggaggagaagaagtctgagctgaggcacaagctgaagtacgtgccacacgagtatatcgagctgatcgagatcgccaggaacagcacccaggaccgcatcctggagatgaaagtgatggagttctttatgaaggtgtacggctataggggcaagcacctgggaggcagccgcaagccagatggagccatctacaccgtgggctcccccatcgactatggcgtgatcgtggatacaaaggcctactccggcggctataatctgcccatcggccaggccgatgagatgcagcggtacgtggaggagaaccagaccagaaataagcacatcaaccctaatgagtggtggaaggtgtatccaagctccgtgacagagttcaagtttctgttcgtgagcggccacttcaagggcaactacaaggcccagctgacccggctgaatcacatcacaaactgtaatggagccgtgctgtccgtggaggagctgctgatcggcggcgagatgatcaaggcaggcaccctgacactggaggaggtgcggagaaagttcaacaatggcgagatcaactttggcggcggcggctcaggcggcggcggctctggaggaggaggaagcggaggaggaggaagcgggggcggcggctctggcggcggcggcagcggaggaggaggatctggaggaggaggatccggcggcggcggcagcgggggaggagggagcggaggaggagggtccggaggaggcggcagccagctggtcaaaagcgaactggaggagaagaagtccgagctgagacataagctgaagtatgtgcctcatgaatacattgaactgattgagatcgcccggaactctacccaggacagaatcctggaaatgaaagtgatggagttctttatgaaagtctatggatacagaggcaagcacctgggcggctctcgcaagcctgacggcgctatctacactgtgggcagcccaattgattacggcgtgatcgtcgatacaaaggcctacagtggaggctataatctgccaatcggacaggcagacgagatgcagcggtatgtggaggaaaatcagactaggaataagcacatcaaccccaacgaatggtggaaggtgtacccttctagcgtgacagagtttaagttcctgttcgtgagcggacactttaagggaaattataaagctcagctgactcggctgaatcatattacaaactgcaatggagccgtgctgagtgtcgaagaactgctgattggaggcgagatgatcaaggccggcaccctgacactggaagaggtgaggcgcaagttcaacaacggagagatcaacttt

SEQ ID NO: 63 - protein, 452 aa, synthetic construct
  REGION 1..452: note = Synthetic Construct
QLVKSELEEKKSELRHKLKYVPHEYIELIEIARNSTQDRILEMKVMEFFMKVYGYRGKHLGGSRKPDGAIYTVGSPIDYGVIVDTKAYSGGYNLPIGQADEMQRYVEENQTRNKHINPNEWWKVYPSSVTEFKFLFVSGHFKGNYKAQLTRLNHITNCNGAVLSVEELLIGGEMIKAGTLTLEEVRRKFNNGEINFGGGGSGGGGSGGGGSGGGGSGGGGSGGGGSGGGGSGGGGSGGGGSGGGGSGGGGSGGGGSQLVKSELEEKKSELRHKLKYVPHEYIELIEIARNSTQDRILEMKVMEFFMKVYGYRGKHLGGSRKPDGAIYTVGSPIDYGVIVDTKAYSGGYNLPIGQADEMQRYVEENQTRNKHINPNEWWKVYPSSVTEFKFLFVSGHFKGNYKAQLTRLNHITNCNGAVLSVEELLIGGEMIKAGTLTLEEVRRKFNNGEINF

SEQ ID NO: 64 - DNA, 528 bp, synthetic construct
  misc_feature 1..528: note = N-terminal domain of TALE63
  source 1..528: mol_type = other DNA
  CDS 1..528
atggactataaggaccacgacggagactacaaggatcatgatattgattacaaagacgatgacgataagatggccccaaagaagaagcggaaggtcggtatccacggagtcccagcagccgtagatttgagaactttgggatattcacagcagcagcaggaaaagatcaagcccaaagtgaggtcgacagtcgcgcagcatcacgaagcgctggtgggtcatgggtttacacatgcccacatcgtagccttgtcgcagcaccctgcagcccttggcacggtcgccgtcaagtaccaggacatgattgcggcgttgccggaagccacacatgaggcgatcgtcggtgtggggaaacagtggagcggagcccgagcgcttgaggccctgttgacggtcgcgggagagctgagagggcctccccttcagctggacacgggccagttgctgaagatcgcgaagcggggaggagtcacggcggtcgaggcggtacacgcgtggcgcaatgcgctcacgggagcacccctcaag

SEQ ID NO: 65 - protein, 176 aa, synthetic construct
  REGION 1..176: note = Synthetic Construct
MDYKDHDGDYKDHDIDYKDDDDKMAPKKKRKVGIHGVPAAVDLRTLGYSQQQQEKIKPKVRSTVAQHHEALVGHGFTHAHIVALSQHPAALGTVAVKYQDMIAALPEATHEAIVGVGKQWSGARALEALLTVAGELRGPPLQLDTGQLLKIAKRGGVTAVEAVHAWRNALTGAPLK

SEQ ID NO: 66 - DNA, 252 bp, synthetic construct
  misc_feature 1..252: note = C-terminal domain of TALE63
  source 1..252: mol_type = other DNA
  CDS 1..252
acccctgagcaggtagtggctattgcatccaacaacgggggcagacccgcactggagtcaatcgtggcccagctttcgaggccggaccccgcgctggccgcactcactaatgatcatcttgtagcgctggcctgcctcggcggacgacccgccttggatgcggtgaagaaggggctcccgcacgcgcctgcattgattaagcggaccaacagaaggatccccgagaggacatcacacagagtggccggttcc

SEQ ID NO: 67 - protein, 84 aa, synthetic construct
  REGION 1..84: note = Synthetic Construct
TPEQVVAIASNNGGRPALESIVAQLSRPDPALAALTNDHLVALACLGGRPALDAVKKGLPHAPALIKRTNRRIPERTSHRVAGS

SEQ ID NO: 68 - DNA, 567 bp, synthetic construct
  misc_feature 1..567: note = N-terminal domain of TALE47
  source 1..567: mol_type = other DNA
  CDS 1..567
atggcttcctcccctccaaagaaaaagagaaaggttgcggccgctgactacaaggatgacgacgataaaagttggaaggacgcaagtggttggtctagaatgcatgcggccccgcgacggcgtgctgcgcaaccctccgacgcttcgccggccgcgcaggtggatctacgcacgctcggctacagtcagcagcagcaagagaagatcaaaccgaaggtgcgttcgacagtggcgcagcaccacgaggcactggtgggccatgggtttacacacgcgcacatcgttgcgctcagccaacacccggcagcgttagggaccgtcgctgtcacgtatcagcacataatcacggcgttgccagaggcgacacacgaagacatcgttggcgtcggcaaacagtggtccggcgcacgcgccctggaggccttgctcacggatgcgggggagttgagaggtccgccgttacagttggacacaggccaacttgtgaagattgcaaaacgtggcggcgtgaccgcaatggaggcagtgcatgcatcgcgcaatgcgctcacgggagcacccctcaag

SEQ ID NO: 69 - protein, 189 aa, synthetic construct
  REGION 1..189: note = Synthetic Construct
MASSPPKKKRKVAAADYKDDDDKSWKDASGWSRMHAAPRRRAAQPSDASPAAQVDLRTLGYSQQQQEKIKPKVRSTVAQHHEALVGHGFTHAHIVALSQHPAALGTVAVTYQHIITALPEATHEDIVGVGKQWSGARALEALLTDAGELRGPPLQLDTGQLVKIAKRGGVTAMEAVHASRNALTGAPLK

SEQ ID NO: 70 - DNA, 204 bp, synthetic construct
  misc_feature 1..204: note = C-terminal domain of TALE47
  source 1..204: mol_type = other DNA
  CDS 1..204
acccctgagcaggtagtggctattgcatccaacaacgggggcagacccgcactggagtcaatcgtggcccagctttcgaggccggaccccgcgctggccgcactcactaatgatcatcttgtagcgctggcctgcctcggcggacgtcctgccatggatgcagtgaaaaagggattgccgcacgcgccggaattgatcagatcc

SEQ ID NO: 71 - protein, 68 aa, synthetic construct
  REGION 1..68: note = Synthetic Construct
TPEQVVAIASNNGGRPALESIVAQLSRPDPALAALTNDHLVALACLGGRPAMDAVKKGLPHAPELIRS

SEQ ID NO: 72 - DNA, 1374 bp, synthetic construct
  misc_feature 1..1374: note = ND1-60-ND1
  source 1..1374: mol_type = other DNA
  CDS 1..1374
cttgttaagggcgaaatggagaaaaagaagtcagatctccgacacaagctgaaacatgtgccacatgagtacattgaactgatagagattgctcaggattccaaacagaaccggctttttgagttcaaggtggtagagtttcttaaggaagtgtatgactacaacgggaaacacctaggcgggtccagaaaacctgacggagctctgtataccaatgggctgaaaaccgactatgggatcatactagacacaaaggcctacaaggatgggtatagcctccctattagccaggccgatgagatgcagcggtacgttgacgaaaacaataaccgcaatgccatcattaaccccaacgagtggtggaaagtctacccgaattccatcctggactttaaattcttattcgtttctggcttctttaaaggcgactataagaaacagttagccagagtgtccaacctgaccaagaggaaaggagctgtcctcagtgtcgaacaattgctccttgggggcgaaaagatcaaggacggatctctgactttagaggacgtaggcgataaattcaacaacgatgagattatcttttacacccgggtgggcggcggcggctcaggcggcggcggctctggaggaggaggaagcggaggaggaggaagcgggggcggcggctctggcggcggcggcagcggaggaggaggatctggaggaggaggatccggcggcggcggcagcgggggaggagggagcggaggaggagggtccggaggaggcggcagcatgaccgcggtcctcgtgaaaggggagatggaaaagaagaagagtgacctgaggcacaaattgaaacacgttcctcacgagtacatcgagctgattgagattgcacaagattcgaagcagaatcgcctctttgagtttaaagtcgtcgaatttctcaaagaagtgtacgattacaatggtaagcatcttggtggatctcgcaagccagatggagccttgtacaccaatggcctgaagactgactatggcattatcctggatacgaaagcgtataaggacggctatagtctgccaatcagccaagcagatgaaatgcagagatacgtggatgaaaacaacaataggaatgccataatcaatcccaatgaatggtggaaggtgtatcccaacagcattctggacttcaagttcctgtttgtatctggtttcttcaagggagactacaagaaacagcttgcacgtgtcagcaacctgacaaaacggaagggtgctgtgttgtcagtggagcagctcttgctaggaggcgagaaaataaaggatggttcactgacactggaagacgtgggagataagttcaacaatgacgagatcatcttc

SEQ ID NO: 73 - protein, 458 aa, synthetic construct
  REGION 1..458: note = Synthetic Construct
LVKGEMEKKKSDLRHKLKHVPHEYIELIEIAQDSKQNRLFEFKVVEFLKEVYDYNGKHLGGSRKPDGALYTNGLKTDYGIILDTKAYKDGYSLPISQADEMQRYVDENNNRNAIINPNEWWKVYPNSILDFKFLFVSGFFKGDYKKQLARVSNLTKRKGAVLSVEQLLLGGEKIKDGSLTLEDVGDKFNNDEIIFYTRVGGGGSGGGGSGGGGSGGGGSGGGGSGGGGSGGGGSGGGGSGGGGSGGGGSGGGGSGGGGSMTAVLVKGEMEKKKSDLRHKLKHVPHEYIELIEIAQDSKQNRLFEFKVVEFLKEVYDYNGKHLGGSRKPDGALYTNGLKTDYGIILDTKAYKDGYSLPISQADEMQRYVDENNNRNAIINPNEWWKVYPNSILDFKFLFVSGFFKGDYKKQLARVSNLTKRKGAVLSVEQLLLGGEKIKDGSLTLEDVGDKFNNDEIIF

SEQ ID NO: 74 - DNA, 1566 bp, synthetic construct
  misc_feature 1..1566: note = ND1-120-ND1
  source 1..1566: mol_type = other DNA
  CDS 1..1566
cttgttaagggcgaaatggagaaaaagaagtcagatctccgacacaagctgaaacatgtgccacatgagtacattgaactgatagagattgctcaggattccaaacagaaccggctttttgagttcaaggtggtagagtttcttaaggaagtgtatgactacaacgggaaacacctaggcgggtccagaaaacctgacggagctctgtataccaatgggctgaaaaccgactatgggatcatactagacacaaaggcctacaaggatgggtatagcctccctattagccaggccgatgagatgcagcggtacgttgacgaaaacaataaccgcaatgccatcattaaccccaacgagtggtggaaagtctacccgaattccatcctggactttaaattcttattcgtttctggcttctttaaaggcgactataagaaacagttagccagagtgtccaacctgaccaagaggaaaggagctgtcctcagtgtcgaacaattgctccttgggggcgaaaagatcaaggacggatctctgactttagaggacgtaggcgataaattcaacaacgatgagattatcttttacacccgggtgggcggcggcggctcaggcggcggcggctctggaggaggaggaagcggaggaggaggaagcgggggcggcggctctggcggcggcggcagcggaggaggaggatctggaggaggaggatccggcggcggcggcagcgggggaggagggagcggaggaggagggtccggaggaggcggcagcatgaccggggtgggcggcggcggctcaggcggcggcggctctggaggaggaggaagcggaggaggaggaagcgggggcggcggctctggcggcggcggcagcggaggaggaggatctggaggaggaggatccggcggcggcggcagcgggggaggagggagcggaggaggagggtccggaggaggcggcagcatgaccgcggtcctcgtgaaaggggagatggaaaagaagaagagtgacctgaggcacaaattgaaacacgttcctcacgagtacatcgagctgattgagattgcacaagattcgaagcagaatcgcctctttgagtttaaagtcgtcgaatttctcaaagaagtgtacgattacaatggtaagcatcttggtggatctcgcaagccagatggagccttgtacaccaatggcctgaagactgactatggcattatcctggatacgaaagcgtataaggacggctatagtctgccaatcagccaagcagatgaaatgcagagatacgtggatgaaaacaacaataggaatgccataatcaatcccaatgaatggtggaaggtgtatcccaacagcattctggacttcaagttcctgtttgtatctggtttcttcaagggagactacaagaaacagcttgcacgtgtcagcaacctgacaaaacggaagggtgctgtgttgtcagtggagcagctcttgctaggaggcgagaaaataaaggatggttcactgacactggaagacgtgggagataagttcaacaatgacgagatcatcttc

SEQ ID NO: 75 - protein, 522 aa, synthetic construct
  REGION 1..522: note = Synthetic Construct
LVKGEMEKKKSDLRHKLKHVPHEYIELIEIAQDSKQNRLFEFKVVEFLKEVYDYNGKHLGGSRKPDGALYTNGLKTDYGIILDTKAYKDGYSLPISQADEMQRYVDENNNRNAIINPNEWWKVYPNSILDFKFLFVSGFFKGDYKKQLARVSNLTKRKGAVLSVEQLLLGGEKIKDGSLTLEDVGDKFNNDEIIFYTRVGGGGSGGGGSGGGGSGGGGSGGGGSGGGGSGGGGSGGGGSGGGGSGGGGSGGGGSGGGGSMTGVGGGGSGGGGSGGGGSGGGGSGGGGSGGGGSGGGGSGGGGSGGGGSGGGGSGGGGSGGGGSMTAVLVKGEMEKKKSDLRHKLKHVPHEYIELIEIAQDSKQNRLFEFKVVEFLKEVYDYNGKHLGGSRKPDGALYTNGLKTDYGIILDTKAYKDGYSLPISQADEMQRYVDENNNRNAIINPNEWWKVYPNSILDFKFLFVSGFFKGDYKKQLARVSNLTKRKGAVLSVEQLLLGGEKIKDGSLTLEDVGDKFNNDEIIF

SEQ ID NO: 76 - DNA, 1758 bp, synthetic construct
  misc_feature 1..1758: note = ND1-180-ND1
  source 1..1758: mol_type = other DNA
  CDS 1..1758
cttgttaagggcgaaatggagaaaaagaagtcagatctccgacacaagctgaaacatgtgccacatgagtacattgaactgatagagattgctcaggattccaaacagaaccggctttttgagttcaaggtggtagagtttcttaaggaagtgtatgactacaacgggaaacacctaggcgggtccagaaaacctgacggagctctgtataccaatgggctgaaaaccgactatgggatcatactagacacaaaggcctacaaggatgggtatagcctccctattagccaggccgatgagatgcagcggtacgttgacgaaaacaataaccgcaatgccatcattaaccccaacgagtggtggaaagtctacccgaattccatcctggactttaaattcttattcgtttctggcttctttaaaggcgactataagaaacagttagccagagtgtccaacctgaccaagaggaaaggagctgtcctcagtgtcgaacaattgctccttgggggcgaaaagatcaaggacggatctctgactttagaggacgtaggcgataaattcaacaacgatgagattatcttttacacccgggtgggcggcggcggctcaggcggcggcggctctggaggaggaggaagcggaggaggaggaagcgggggcggcggctctggcggcggcggcagcggaggaggaggatctggaggaggaggatccggcggcggcggcagcgggggaggagggagcggaggaggagggtccggaggaggcggcagcatgaccggggtgggcggcggcggctcaggcggcggcggctctggaggaggaggaagcggaggaggaggaagcgggggcggcggctctggcggcggcggcagcggaggaggaggatctggaggaggaggatccggcggcggcggcagcgggggaggagggagcggaggaggagggtccggaggaggcggcagcatgaccggggtgggcggcggcggctcaggcggcggcggctctggaggaggaggaagcggaggaggaggaagcgggggcggcggctctggcggcggcggcagcggaggaggaggatctggaggaggaggatccggcggcggcggcagcgggggaggagggagcggaggaggagggtccggaggaggcggcagcatgaccgcggtcctcgtgaaaggggagatggaaaagaagaagagtgacctgaggcacaaattgaaacacgttcctcacgagtacatcgagctgattgagattgcacaagattcgaagcagaatcgcctctttgagtttaaagtcgtcgaatttctcaaagaagtgtacgattacaatggtaagcatcttggtggatctcgcaagccagatggagccttgtacaccaatggcctgaagactgactatggcattatcctggatacgaaagcgtataaggacggctatagtctgccaatcagccaagcagatgaaatgcagagatacgtggatgaaaacaacaataggaatgccataatcaatcccaatgaatggtggaaggtgtatcccaacagcattctggacttcaagttcctgtttgtatctggtttcttcaagggagactacaagaaacagcttgcacgtgtcagcaacctgacaaaacggaagggtgctgtgttgtcagtggagcagctcttgctaggaggcgagaaaataaaggatggttcactgacactggaagacgtgggagataagttcaacaatgacgagatcatcttc

SEQ ID NO: 77 - protein, 586 aa, synthetic construct
  REGION 1..586: note = Synthetic Construct
LVKGEMEKKKSDLRHKLKHVPHEYIELIEIAQDSKQNRLFEFKVVEFLKEVYDYNGKHLGGSRKPDGALYTNGLKTDYGIILDTKAYKDGYSLPISQADEMQRYVDENNNRNAIINPNEWWKVYPNSILDFKFLFVSGFFKGDYKKQLARVSNLTKRKGAVLSVEQLLLGGEKIKDGSLTLEDVGDKFNNDEIIFYTRVGGGGSGGGGSGGGGSGGGGSGGGGSGGGGSGGGGSGGGGSGGGGSGGGGSGGGGSGGGGSMTGVGGGGSGGGGSGGGGSGGGGSGGGGSGGGGSGGGGSGGGGSGGGGSGGGGSGGGGSGGGGSMTGVGGGGSGGGGSGGGGSGGGGSGGGGSGGGGSGGGGSGGGGSGGGGSGGGGSGGGGSGGGGSMTAVLVKGEMEKKKSDLRHKLKHVPHEYIELIEIAQDSKQNRLFEFKVVEFLKEVYDYNGKHLGGSRKPDGALYTNGLKTDYGIILDTKAYKDGYSLPISQADEMQRYVDENNNRNAIINPNEWWKVYPNSILDFKFLFVSGFFKGDYKKQLARVSNLTKRKGAVLSVEQLLLGGEKIKDGSLTLEDVGDKFNNDEIIF

SEQ ID NO: 78 - DNA, 1479 bp, synthetic construct
  misc_feature 1..1479: note = ND1-95-ND1
  source 1..1479: mol_type = other DNA
  CDS 1..1479
cttgttaagggcgaaatggagaaaaagaagtcagatctccgacacaagctgaaacatgtgccacatgagtacattgaactgatagagattgctcaggattccaaacagaaccggctttttgagttcaaggtggtagagtttcttaaggaagtgtatgactacaacgggaaacacctaggcgggtccagaaaacctgacggagctctgtataccaatgggctgaaaaccgactatgggatcatactagacacaaaggcctacaaggatgggtatagcctccctattagccaggccgatgagatgcagcggtacgttgacgaaaacaataaccgcaatgccatcattaaccccaacgagtggtggaaagtctacccgaattccatcctggactttaaattcttattcgtttctggcttctttaaaggcgactataagaaacagttagccagagtgtccaacctgaccaagaggaaaggagctgtcctcagtgtcgaacaattgctccttgggggcgaaaagatcaaggacggatctctgactttagaggacgtaggcgataaattcaacaacgatgagattatcttttacacccgggtgggaagcggatccggatctggaagcatcaccaggaccacaaaccctcgcaatgtggtgccaaagatctacatgtccgccggctctatccctctgaccacacacatcacaaacagcatccagccaaccctgtggacaatcggatccatcaatggagtggcaccactggccaagtctatcaagctgggcatccctgtgaccggcagcgcctacacagaccagaccacagccatggtgcggaagaaggtgagcgtgttcatgggcagcggatctggaagcggatctagcatgaccgcggtcctcgtgaaaggggagatggaaaagaagaagagtgacctgaggcacaaattgaaacacgttcctcacgagtacatcgagctgattgagattgcacaagattcgaagcagaatcgcctctttgagtttaaagtcgtcgaatttctcaaagaagtgtacgattacaatggtaagcatcttggtggatctcgcaagccagatggagccttgtacaccaatggcctgaagactgactatggcattatcctggatacgaaagcgtataaggacggctatagtctgccaatcagccaagcagatgaaatgcagagatacgtggatgaaaacaacaataggaatgccataatcaatcccaatgaatggtggaaggtgtatcccaacagcattctggacttcaagttcctgtttgtatctggtttcttcaagggagactacaagaaacagcttgcacgtgtcagcaacctgacaaaacggaagggtgctgtgttgtcagtggagcagctcttgctaggaggcgagaaaataaaggatggttcactgacactggaagacgtgggagataagttcaacaatgacgagatcatcttc

SEQ ID NO: 79 - protein, 493 aa, synthetic construct
  REGION 1..493: note = Synthetic Construct
LVKGEMEKKKSDLRHKLKHVPHEYIELIEIAQDSKQNRLFEFKVVEFLKEVYDYNGKHLGGSRKPDGALYTNGLKTDYGIILDTKAYKDGYSLPISQADEMQRYVDENNNRNAIINPNEWWKVYPNSILDFKFLFVSGFFKGDYKKQLARVSNLTKRKGAVLSVEQLLLGGEKIKDGSLTLEDVGDKFNNDEIIFYTRVGSGSGSGSITRTTNPRNVVPKIYMSAGSIPLTTHITNSIQPTLWTIGSINGVAPLAKSIKLGIPVTGSAYTDQTTAMVRKKVSVFMGSGSGSGSSMTAVLVKGEMEKKKSDLRHKLKHVPHEYIELIEIAQDSKQNRLFEFKVVEFLKEVYDYNGKHLGGSRKPDGALYTNGLKTDYGIILDTKAYKDGYSLPISQADEMQRYVDENNNRNAIINPNEWWKVYPNSILDFKFLFVSGFFKGDYKKQLARVSNLTKRKGAVLSVEQLLLGGEKIKDGSLTLEDVGDKFNNDEIIF

SEQ ID NO: 80 - DNA, 1350 bp, synthetic construct
  misc_feature 1..1350: note = ND2-60-ND2
  source 1..1350: mol_type = other DNA
  CDS 1..1350
attgttaagagcagcattgagatgagcaaggccaatatgagggataacctacagatgctcccacacgactacatcgagcttatcgagatctctcaggatccttatcaaaaccgcatcttcgaaatgaaagtgatggatctgtttatcaacgaatatggcttcagtgggtcacatctgggaggctccagaaaaccagatggagccatgtatgcccatgggtttggggtgatcgtggacactaaggcgtataaggatggatacaatctccccatatcccaggctgacgaaatggagcgctatgtcagggaaaacatcgaccggaatgagcacgtgaattccaataggtggtggaatatttttccggaagataccaatgagtacaagttcttgtttgtgtctgggttcttcaagggcaatttcgagaagcagctagaacggatttccatcgacacaggggttcaaggaggagctctgtcagtggagcacctgctgctgggggctgaatacataaaacgaggcattcttacactgtatgacttcaagaattcgtttctgaacaaagagatccagttctacacccgggtgggcggcggcggctcaggcggcggcggctctggaggaggaggaagcggaggaggaggaagcgggggcggcggctctggcggcggcggcagcggaggaggaggatctggaggaggaggatccggcggcggcggcagcgggggaggagggagcggaggaggagggtccggaggaggcggcagcatgaccgcggtcattgtgaagtctagtatcgaaatgtccaaagccaatatgcgcgacaatctccagatgcttccccatgactatatcgaactgatcgaaatctcccaagacccttaccagaaccggatatttgagatgaaggtaatggacctgttcattaacgagtatggctttagcggcagtcatctcggtggaagcaggaagcctgatggtgccatgtacgctcacggatttggcgtcattgtcgataccaaagcatacaaggatgggtacaacttgcccataagtcaggccgatgagatggaaagatacgtgagagagaacattgaccgtaacgagcacgtcaatagcaaccgatggtggaacatctttccagaggataccaacgaatacaaattcctctttgtgtcaggtttctttaagggcaactttgaaaaacagcttgagcggatctcaattgacactggcgtacaaggtggcgcattatctgttgaacacttgttactgggagcagagtatattaaaagaggtatattgacgctctacgacttcaaaaactctttcctgaataaggagattcagttc

SEQ ID NO: 81 - protein, 450 aa, synthetic construct
  REGION 1..450: note = Synthetic Construct
IVKSSIEMSKANMRDNLQMLPHDYIELIEISQDPYQNRIFEMKVMDLFINEYGFSGSHLGGSRKPDGAMYAHGFGVIVDTKAYKDGYNLPISQADEMERYVRENIDRNEHVNSNRWWNIFPEDTNEYKFLFVSGFFKGNFEKQLERISIDTGVQGGALSVEHLLLGAEYIKRGILTLYDFKNSFLNKEIQFYTRVGGGGSGGGGSGGGGSGGGGSGGGGSGGGGSGGGGSGGGGSGGGGSGGGGSGGGGSGGGGSMTAVIVKSSIEMSKANMRDNLQMLPHDYIELIEISQDPYQNRIFEMKVMDLFINEYGFSGSHLGGSRKPDGAMYAHGFGVIVDTKAYKDGYNLPISQADEMERYVRENIDRNEHVNSNRWWNIFPEDTNEYKFLFVSGFFKGNFEKQLERISIDTGVQGGALSVEHLLLGAEYIKRGILTLYDFKNSFLNKEIQF

SEQ ID NO: 82 - DNA, 1542 bp, synthetic construct
  misc_feature 1..1542: note = ND2-120-ND2
  source 1..1542: mol_type = other DNA
  CDS 1..1542
attgttaagagcagcattgagatgagcaaggccaatatgagggataacctacagatgctcccacacgactacatcgagcttatcgagatctctcaggatccttatcaaaaccgcatcttcgaaatgaaagtgatggatctgtttatcaacgaatatggcttcagtgggtcacatctgggaggctccagaaaaccagatggagccatgtatgcccatgggtttggggtgatcgtggacactaaggcgtataaggatggatacaatctccccatatcccaggctgacgaaatggagcgctatgtcagggaaaacatcgaccggaatgagcacgtgaattccaataggtggtggaatatttttccggaagataccaatgagtacaagttcttgtttgtgtctgggttcttcaagggcaatttcgagaagcagctagaacggatttccatcgacacaggggttcaaggaggagctctgtcagtggagcacctgctgctgggggctgaatacataaaacgaggcattcttacactgtatgacttcaagaattcgtttctgaacaaagagatccagttctacacccgggtgggcggcggcggctcaggcggcggcggctctggaggaggaggaagcggaggaggaggaagcgggggcggcggctctggcggcggcggcagcggaggaggaggatctggaggaggaggatccggcggcggcggcagcgggggaggagggagcggaggaggagggtccggaggaggcggcagcatgaccggggtgggcggcggcggctcaggcggcggcggctctggaggaggaggaagcggaggaggaggaagcgggggcggcggctctggcggcggcggcagcggaggaggaggatctggaggaggaggatccggcggcggcggcagcgggggaggagggagcggaggaggagggtccggaggaggcggcagcatgaccgcggtcattgtgaagtctagtatcgaaatgtccaaagccaatatgcgcgacaatctccagatgcttccccatgactatatcgaactgatcgaaatctcccaagacccttaccagaaccggatatttgagatgaaggtaatggacctgttcattaacgagtatggctttagcggcagtcatctcggtggaagcaggaagcctgatggtgccatgtacgctcacggatttggcgtcattgtcgataccaaagcatacaaggatgggtacaacttgcccataagtcaggccgatgagatggaaagatacgtgagagagaacattgaccgtaacgagcacgtcaatagcaaccgatggtggaacatctttccagaggataccaacgaatacaaattcctctttgtgtcaggtttctttaagggcaactttgaaaaacagcttgagcggatctcaattgacactggcgtacaaggtggcgcattatctgttgaacacttgttactgggagcagagtatattaaaagaggtatattgacgctctacgacttcaaaaactctttcctgaataaggagattcagttc

SEQ ID NO: 83 - protein, 514 aa, synthetic construct
  REGION 1..514: note = Synthetic Construct
IVKSSIEMSKANMRDNLQMLPHDYIELIEISQDPYQNRIFEMKVMDLFINEYGFSGSHLGGSRKPDGAMYAHGFGVIVDTKAYKDGYNLPISQADEMERYVRENIDRNEHVNSNRWWNIFPEDTNEYKFLFVSGFFKGNFEKQLERISIDTGVQGGALSVEHLLLGAEYIKRGILTLYDFKNSFLNKEIQFYTRVGGGGSGGGGSGGGGSGGGGSGGGGSGGGGSGGGGSGGGGSGGGGSGGGGSGGGGSGGGGSMTGVGGGGSGGGGSGGGGSGGGGSGGGGSGGGGSGGGGSGGGGSGGGGSGGGGSGGGGSGGGGSMTAVIVKSSIEMSKANMRDNLQMLPHDYIELIEISQDPYQNRIFEMKVMDLFINEYGFSGSHLGGSRKPDGAMYAHGFGVIVDTKAYKDGYNLPISQADEMERYVRENIDRNEHVNSNRWWNIFPEDTNEYKFLFVSGFFKGNFEKQLERISIDTGVQGGALSVEHLLLGAEYIKRGILTLYDFKNSFLNKEIQF

SEQ ID NO: 84 - DNA, 1734 bp, synthetic construct
  misc_feature 1..1734: note = ND2-180-ND2
  source 1..1734: mol_type = other DNA
  CDS 1..1734
attgttaagagcagcattgagatgagcaaggccaatatgagggataacctacagatgctcccacacgactacatcgagcttatcgagatctctcaggatccttatcaaaaccgcatcttcgaaatgaaagtgatggatctgtttatcaacgaatatggcttcagtgggtcacatctgggaggctccagaaaaccagatggagccatgtatgcccatgggtttggggtgatcgtggacactaaggcgtataaggatggatacaatctccccatatcccaggctgacgaaatggagcgctatgtcagggaaaacatcgaccggaatgagcacgtgaattccaataggtggtggaatatttttccggaagataccaatgagtacaagttcttgtttgtgtctgggttcttcaagggcaatttcgagaagcagctagaacggatttccatcgacacaggggttcaaggaggagctctgtcagtggagcacctgctgctgggggctgaatacataaaacgaggcattcttacactgtatgacttcaagaattcgtttctgaacaaagagatccagttctacacccgggtgggcggcggcggctcaggcggcggcggctctggaggaggaggaagcggaggaggaggaagcgggggcggcggctctggcggcggcggcagcggaggaggaggatctggaggaggaggatccggcggcggcggcagcgggggaggagggagcggaggaggagggtccggaggaggcggcagcatgaccggggtgggcggcggcggctcaggcggcggcggctctggaggaggaggaagcggaggaggaggaagcgggggcggcggctctggcggcggcggcagcggaggaggaggatctggaggaggaggatccggcggcggcggcagcgggggaggagggagcggaggaggagggtccggaggaggcggcagcatgaccggggtgggcggcggcggctcaggcggcggcggctctggaggaggaggaagcggaggaggaggaagcgggggcggcggctctggcggcggcggcagcggaggaggaggatctggaggaggaggatccggcggcggcggcagcgggggaggagggagcggaggaggagggtccggaggaggcggcagcatgaccgcggtcattgtgaagtctagtatcgaaatgtccaaagccaatatgcgcgacaatctccagatgcttccccatgactatatcgaactgatcgaaatctcccaagacccttaccagaaccggatatttgagatgaaggtaatggacctgttcattaacgagtatggctttagcggcagtcatctcggtggaagcaggaagcctgatggtgccatgtacgctcacggatttggcgtcattgtcgataccaaagcatacaaggatgggtacaacttgcccataagtcaggccgatgagatggaaagatacgtgagagagaacattgaccgtaacgagcacgtcaatagcaaccgatggtggaacatctttccagaggataccaacgaatacaaattcctctttgtgtcaggtttctttaagggcaactttgaaaaacagcttgagcggatctcaattgacactggcgtacaaggtggcgcattatctgttgaacacttgttactgggagcagagtatattaaaagaggtatattgacgctctacgacttcaaaaactctttcctgaataaggagattcagttc

SEQ ID NO: 85 - protein, 578 aa, synthetic construct
  REGION 1..578: note = Synthetic Construct
IVKSSIEMSKANMRDNLQMLPHDYIELIEISQDPYQNRIFEMKVMDLFINEYGFSGSHLGGSRKPDGAMYAHGFGVIVDTKAYKDGYNLPISQADEMERYVRENIDRNEHVNSNRWWNIFPEDTNEYKFLFVSGFFKGNFEKQLERISIDTGVQGGALSVEHLLLGAEYIKRGILTLYDFKNSFLNKEIQFYTRVGGGGSGGGGSGGGGSGGGGSGGGGSGGGGSGGGGSGGGGSGGGGSGGGGSGGGGSGGGGSMTGVGGGGSGGGGSGGGGSGGGGSGGGGSGGGGSGGGGSGGGGSGGGGSGGGGSGGGGSGGGGSMTGVGGGGSGGGGSGGGGSGGGGSGGGGSGGGGSGGGGSGGGGSGGGGSGGGGSGGGGSGGGGSMTAVIVKSSIEMSKANMRDNLQMLPHDYIELIEISQDPYQNRIFEMKVMDLFINEYGFSGSHLGGSRKPDGAMYAHGFGVIVDTKAYKDGYNLPISQADEMERYVRENIDRNEHVNSNRWWNIFPEDTNEYKFLFVSGFFKGNFEKQLERISIDTGVQGGALSVEHLLLGAEYIKRGILTLYDFKNSFLNKEIQF

SEQ ID NO: 86 - DNA, 1455 bp, synthetic construct
  misc_feature 1..1455: note = ND2-95-ND2
  source 1..1455: mol_type = other DNA
  CDS 1..1455
attgttaagagcagcattgagatgagcaaggccaatatgagggataacctacagatgctcccacacgactacatcgagcttatcgagatctctcaggatccttatcaaaaccgcatcttcgaaatgaaagtgatggatctgtttatcaacgaatatggcttcagtgggtcacatctgggaggctccagaaaaccagatggagccatgtatgcccatgggtttggggtgatcgtggacactaaggcgtataaggatggatacaatctccccatatcccaggctgacgaaatggagcgctatgtcagggaaaacatcgaccggaatgagcacgtgaattccaataggtggtggaatatttttccggaagataccaatgagtacaagttcttgtttgtgtctgggttcttcaagggcaatttcgagaagcagctagaacggatttccatcgacacaggggttcaaggaggagctctgtcagtggagcacctgctgctgggggctgaatacataaaacgaggcattcttacactgtatgacttcaagaattcgtttctgaacaaagagatccagttctacacccgggtgggaagcggatccggatctggaagcatcaccaggaccacaaaccctcgcaatgtggtgccaaagatctacatgtccgccggctctatccctctgaccacacacatcacaaacagcatccagccaaccctgtggacaatcggatccatcaatggagtggcaccactggccaagtctatcaagctgggcatccctgtgaccggcagcgcctacacagaccagaccacagccatggtgcggaagaaggtgagcgtgttcatgggcagcggatctggaagcggatctagcatgaccgcggtcattgtgaagtctagtatcgaaatgtccaaagccaatatgcgcgacaatctccagatgcttccccatgactatatcgaactgatcgaaatctcccaagacccttaccagaaccggatatttgagatgaaggtaatggacctgttcattaacgagtatggctttagcggcagtcatctcggtggaagcaggaagcctgatggtgccatgtacgctcacggatttggcgtcattgtcgataccaaagcatacaaggatgggtacaacttgcccataagtcaggccgatgagatggaaagatacgtgagagagaacattgaccgtaacgagcacgtcaatagcaaccgatggtggaacatctttccagaggataccaacgaatacaaattcctctttgtgtcaggtttctttaagggcaactttgaaaaacagcttgagcggatctcaattgacactggcgtacaaggtggcgcattatctgttgaacacttgttactgggagcagagtatattaaaagaggtatattgacgctctacgacttcaaaaactctttcctgaataaggagattcagttc

SEQ ID NO: 87 - protein, 485 aa, synthetic construct
  REGION 1..485: note = Synthetic Construct
IVKSSIEMSKANMRDNLQMLPHDYIELIEISQDPYQNRIFEMKVMDLFINEYGFSGSHLGGSRKPDGAMYAHGFGVIVDTKAYKDGYNLPISQADEMERYVRENIDRNEHVNSNRWWNIFPEDTNEYKFLFVSGFFKGNFEKQLERISIDTGVQGGALSVEHLLLGAEYIKRGILTLYDFKNSFLNKEIQFYTRVGSGSGSGSITRTTNPRNVVPKIYMSAGSIPLTTHITNSIQPTLWTIGSINGVAPLAKSIKLGIPVTGSAYTDQTTAMVRKKVSVFMGSGSGSGSSMTAVIVKSSIEMSKANMRDNLQMLPHDYIELIEISQDPYQNRIFEMKVMDLFINEYGFSGSHLGGSRKPDGAMYAHGFGVIVDTKAYKDGYNLPISQADEMERYVRENIDRNEHVNSNRWWNIFPEDTNEYKFLFVSGFFKGNFEKQLERISIDTGVQGGALSVEHLLLGAEYIKRGILTLYDFKNSFLNKEIQF

SEQ ID NO: 88 - DNA, 1497 bp, synthetic construct
  misc_feature 1..1497: note = ND1-GSSx32-ND1
  source 1..1497: mol_type = other DNA
  CDS 1..1497
cttgttaagggcgaaatggagaaaaagaagtcagatctccgacacaagctgaaacatgtgccacatgagtacattgaactgatagagattgctcaggattccaaacagaaccggctttttgagttcaaggtggtagagtttcttaaggaagtgtatgactacaacgggaaacacctaggcgggtccagaaaacctgacggagctctgtataccaatgggctgaaaaccgactatgggatcatactagacacaaaggcctacaaggatgggtatagcctccctattagccaggccgatgagatgcagcggtacgttgacgaaaacaataaccgcaatgccatcattaaccccaacgagtggtggaaagtctacccgaattccatcctggactttaaattcttattcgtttctggcttctttaaaggcgactataagaaacagttagccagagtgtccaacctgaccaagaggaaaggagctgtcctcagtgtcgaacaattgctccttgggggcgaaaagatcaaggacggatctctgactttagaggacgtaggcgataaattcaacaacgatgagattatcttttacacccgggtggggtctagtggctccagcggatcaagtggcagctccgggtctagtggctccagcggatcaagtgggagttctggcagctcaggatctagtggcagctccgggtctagtggctccagcggatcaagtgggagttctggcagctcaggatctagtggcagctccgggtctagtggctccagcggatcaagtgggagttctggcagctcaggatctagtggcagctccgggtctagtggctccagcggatcaagtgggagttctggcagctcaggatctagtggcagctccggaggaggcggcagcatgaccgcggtcctcgtgaaaggggagatggaaaagaagaagagtgacctgaggcacaaattgaaacacgttcctcacgagtacatcgagctgattgagattgcacaagattcgaagcagaatcgcctctttgagtttaaagtcgtcgaatttctcaaagaagtgtacgattacaatggtaagcatcttggtggatctcgcaagccagatggagccttgtacaccaatggcctgaagactgactatggcattatcctggatacgaaagcgtataaggacggctatagtctgccaatcagccaagcagatgaaatgcagagatacgtggatgaaaacaacaataggaatgccataatcaatcccaatgaatggtggaaggtgtatcccaacagcattctggacttcaagttcctgtttgtatctggtttcttcaagggagactacaagaaacagcttgcacgtgtcagcaacctgacaaaacggaagggtgctgtgttgtcagtggagcagctcttgctaggaggcgagaaaataaaggatggttcactgacactggaagacgtgggagataagttcaacaatgacgagatcatcttc

SEQ ID NO: 89 - protein, 499 aa, synthetic construct
  REGION 1..499: note = Synthetic Construct
LVKGEMEKKKSDLRHKLKHVPHEYIELIEIAQDSKQNRLFEFKVVEFLKEVYDYNGKHLGGSRKPDGALYTNGLKTDYGIILDTKAYKDGYSLPISQADEMQRYVDENNNRNAIINPNEWWKVYPNSILDFKFLFVSGFFKGDYKKQLARVSNLTKRKGAVLSVEQLLLGGEKIKDGSLTLEDVGDKFNNDEIIFYTRVGSSGSSGSSGSSGSSGSSGSSGSSGSSGSSGSSGSSGSSGSSGSSGSSGSSGSSGSSGSSGSSGSSGSSGSSGSSGSSGSSGSSGSSGSSGSSGSSGGGGSMTAVLVKGEMEKKKSDLRHKLKHVPHEYIELIEIAQDSKQNRLFEFKVVEFLKEVYDYNGKHLGGSRKPDGALYTNGLKTDYGIILDTKAYKDGYSLPISQADEMQRYVDENNNRNAIINPNEWWKVYPNSILDFKFLFVSGFFKGDYKKQLARVSNLTKRKGAVLSVEQLLLGGEKIKDGSLTLEDVGDKFNNDEIIF

SEQ ID NO: 90 - DNA, 1485 bp, synthetic construct
  misc_feature 1..1485: note = ND1-SAGGx24-ND1
  source 1..1485: mol_type = other DNA
  CDS 1..1485
cttgttaagggcgaaatggagaaaaagaagtcagatctccgacacaagctgaaacatgtgccacatgagtacattgaactgatagagattgctcaggattccaaacagaaccggctttttgagttcaaggtggtagagtttcttaaggaagtgtatgactacaacgggaaacacctaggcgggtccagaaaacctgacggagctctgtataccaatgggctgaaaaccgactatgggatcatactagacacaaaggcctacaaggatgggtatagcctccctattagccaggccgatgagatgcagcggtacgttgacgaaaacaataaccgcaatgccatcattaaccccaacgagtggtggaaagtctacccgaattccatcctggactttaaattcttattcgtttctggcttctttaaaggcgactataagaaacagttagccagagtgtccaacctgaccaagaggaaaggagctgtcctcagtgtcgaacaattgctccttgggggcgaaaagatcaaggacggatctctgactttagaggacgtaggcgataaattcaacaacgatgagattatcttttacacccgggtgtctgctggcgggtccgccgggggcagtgctggcggatctgctggcgggtccgccgggggcagtgctggcggatctgctggcgggtccgccgggggcagtgctggcggatctgctggcgggtccgccgggggcagtgctggcggatctgctggcgggtccgccgggggcagtgctggcggatctgctggcgggtccgccgggggcagtgctggcggatctgctggcgggtccgccgggggcagtgctggcggatctgctggcgggtccgccgggggcagtgctggcggatccatgaccgcggtcctcgtgaaaggggagatggaaaagaagaagagtgacctgaggcacaaattgaaacacgttcctcacgagtacatcgagctgattgagattgcacaagattcgaagcagaatcgcctctttgagtttaaagtcgtcgaatttctcaaagaagtgtacgattacaatggtaagcatcttggtggatctcgcaagccagatggagccttgtacaccaatggcctgaagactgactatggcattatcctggatacgaaagcgtataaggacggctatagtctgccaatcagccaagcagatgaaatgcagagatacgtggatgaaaacaacaataggaatgccataatcaatcccaatgaatggtggaaggtgtatcccaacagcattctggacttcaagttcctgtttgtatctggtttcttcaagggagactacaagaaacagcttgcacgtgtcagcaacctgacaaaacggaagggtgctgtgttgtcagtggagcagctcttgctaggaggcgagaaaataaaggatggttcactgacactggaagacgtgggagataagttcaacaatgacgagatcatcttc

SEQ ID NO: 91 - protein, 495 aa, synthetic construct
  REGION 1..495: note = Synthetic Construct
LVKGEMEKKKSDLRHKLKHVPHEYIELIEIAQDSKQNRLFEFKVVEFLKEVYDYNGKHLGGSRKPDGALYTNGLKTDYGIILDTKAYKDGYSLPISQADEMQRYVDENNNRNAIINPNEWWKVYPNSILDFKFLFVSGFFKGDYKKQLARVSNLTKRKGAVLSVEQLLLGGEKIKDGSLTLEDVGDKFNNDEIIFYTRVSAGGSAGGSAGGSAGGSAGGSAGGSAGGSAGGSAGGSAGGSAGGSAGGSAGGSAGGSAGGSAGGSAGGSAGGSAGGSAGGSAGGSAGGSAGGSAGGSMTAVLVKGEMEKKKSDLRHKLKHVPHEYIELIEIAQDSKQNRLFEFKVVEFLKEVYDYNGKHLGGSRKPDGALYTNGLKTDYGIILDTKAYKDGYSLPISQADEMQRYVDENNNRNAIINPNEWWKVYPNSILDFKFLFVSGFFKGDYKKQLARVSNLTKRKGAVLSVEQLLLGGEKIKDGSLTLEDVGDKFNNDEIIF

SEQ ID NO: 92 - DNA, 1482 bp, synthetic construct
  misc_feature 1..1482: note = ND1-GGGGSx19-ND1
  source 1..1482: mol_type = other DNA
  CDS 1..1482
cttgttaagggcgaaatggagaaaaagaagtcagatctccgacacaagctgaaacatgtgccacatgagtacattgaactgatagagattgctcaggattccaaacagaaccggctttttgagttcaaggtggtagagtttcttaaggaagtgtatgactacaacgggaaacacctaggcgggtccagaaaacctgacggagctctgtataccaatgggctgaaaaccgactatgggatcatactagacacaaaggcctacaaggatgggtatagcctccctattagccaggccgatgagatgcagcggtacgttgacgaaaacaataaccgcaatgccatcattaaccccaacgagtggtggaaagtctacccgaattccatcctggactttaaattcttattcgtttctggcttctttaaaggcgactataagaaacagttagccagagtgtccaacctgaccaagaggaaaggagctgtcctcagtgtcgaacaattgctccttgggggcgaaaagatcaaggacggatctctgactttagaggacgtaggcgataaattcaacaacgatgagattatcttttacacccgggtggggggcggagggtctggcggagggggctctggagggggcggatccgggggcggagggtctggcggagggggctctggagggggcggatccgggggcggagggtctggcggagggggctctggagggggcggatccgggggcggagggtctggcggagggggctctggagggggcggatccgggggcggagggtctggcggagggggctctggagggggcggatccgggggcggagggtctggcggagggggctctggagggggcggatcagggggcggagggtccggaatgaccgcggtcctcgtgaaaggggagatggaaaagaagaagagtgacctgaggcacaaattgaaacacgttcctcacgagtacatcgagctgattgagattgcacaagattcgaagcagaatcgcctctttgagtttaaagtcgtcgaatttctcaaagaagtgtacgattacaatggtaagcatcttggtggatctcgcaagccagatggagccttgtacaccaatggcctgaagactgactatggcattatcctggatacgaaagcgtataaggacggctatagtctgccaatcagccaagcagatgaaatgcagagatacgtggatgaaaacaacaataggaatgccataatcaatcccaatgaatggtggaaggtgtatcccaacagcattctggacttcaagttcctgtttgtatctggtttcttcaagggagactacaagaaacagcttgcacgtgtcagcaacctgacaaaacggaagggtgctgtgttgtcagtggagcagctcttgctaggaggcgagaaaataaaggatggttcactgacactggaagacgtgggagataagttcaacaatgacgagatcatcttc

SEQ ID NO: 93 - protein, 494 aa, synthetic construct
  REGION 1..494: note = Synthetic Construct
LVKGEMEKKKSDLRHKLKHVPHEYIELIEIAQDSKQNRLFEFKVVEFLKEVYDYNGKHLGGSRKPDGALYTNGLKTDYGIILDTKAYKDGYSLPISQADEMQRYVDENNNRNAIINPNEWWKVYPNSILDFKFLFVSGFFKGDYKKQLARVSNLTKRKGAVLSVEQLLLGGEKIKDGSLTLEDVGDKFNNDEIIFYTRVGGGGSGGGGSGGGGSGGGGSGGGGSGGGGSGGGGSGGGGSGGGGSGGGGSGGGGSGGGGSGGGGSGGGGSGGGGSGGGGSGGGGSGGGGSGGGGSGMTAVLVKGEMEKKKSDLRHKLKHVPHEYIELIEIAQDSKQNRLFEFKVVEFLKEVYDYNGKHLGGSRKPDGALYTNGLKTDYGIILDTKAYKDGYSLPISQADEMQRYVDENNNRNAIINPNEWWKVYPNSILDFKFLFVSGFFKGDYKKQLARVSNLTKRKGAVLSVEQLLLGGEKIKDGSLTLEDVGDKFNNDEIIF

SEQ ID NO: 94 - DNA, 237 bp, synthetic construct
  misc_feature 1..237: note = EGxAPCxFP
  source 1..237: mol_type = other DNA
ctcgatgctgttcccaggtactgttgttggctgttggtgaggaaggtgaagcactcagttgccttctcgggcctcggcgccccctatgtacgcctccctgggctcgggtccggtcgcccctttgcccgcttctgtaccaccctcagttctcgggtcctggagcaccggcggcagcaggagctgcgtccggcaggagacgaagagcccgggcggcgctcgtacttctggccactgggc

SEQ ID NO: 95 - DNA, 433 bp, synthetic construct
  misc_feature 1..433: note = EGxRosa26xFP
  source 1..433: mol_type = other DNA
gggagaaggccgcaccctactcggctgggggaggggagtgccgcaatacctttctgggagttctctgctgcctcctgtcttctaaagaccgccccgggactggaaggatcccttccccctttcccctcgtgatctgcaagtcgaggctttctgggagatgggcgggagtcttctgggcaggcttgagggctaacctggtgcgtgggcgttgtcctgcaggggaattgaactggtgtaaaattggaagggtgagaattcccacggattttcgtttgtgtcgggaggtgattgtaataggggcaaaggagggaaatgggagactaggtgctcgcctggggttttgtgcagcaaaactacaggttattattaataagccttggagtatttttcatcgagttggattaaggtcatgctcacccgagttttatgctca

SEQ ID NO: 96 - DNA, 721 bp, synthetic construct
  misc_feature 1..721: note = EGxHPRT1xFP
  source 1..721: mol_type = other DNA
gacacacatatgcacttgcatttgcccccacaatgctcaaacatactcaatgtgtagagtagaaactgcgtagactagtctctgatgtttaaagtatttttgccacatttgtcatacctctttaaattgttatctttttctacttgtgacctgaaggaagaggattatagtttattacaaaaatataaaattaactgcccttcataccctctcatacccaaattcctctggcgaactaaggcttattttctaaattttgttaaatatggatatcttatgctctgatttgaaacagctgtctttctttttcagattagtgatgatgaaccaggctatgacctagatttattttgtattcctaatcactatgtcgaggatttggaaaaggtgtttattcctcatggagtgattatggacaggtaagtaagatcttaattgaaggggctggagagatggctcagcggttaagagcactgactgctcttccagaggttctgagttcaattcccagcaaccacatgatggctcacaaccatccctaatgagatctggtgccctcttctggcctgcagggacacatgcagacagaacagatcttaattgaagttttatgggtttattttagatgtgtctgtgtatgtttgtgataggcatgtatttgatacatatgtataatgtatatatttatgtaaaagctagagaaggacattgggtgccatac

SEQ ID NO: 97 - protein, 585 aa, Bacillus sp. SGD-V-76
MATKRVVRTFGWIQNPGKFENLKRTVQVFDENSKVYKEVRDIKIPNLVKDKDVRTTLIAAMNRLENYYSYKELVGTGTSVRAQAPCDAIIQAAIQDQGNKKGYIDNWSSDGFVRWAHALGFLEYNSDKDSFYLTDIGLEYSRSTDDSLNEKIILIEALSSYPPAIRILTLLENGEHLTKFDLGKQLGFSGESGFTSLPQNLFLDALANAPSSPPTIKNSIRSDWEGSADKYARMISGWLVKMGLVAQGRKNFVVPTVGGSTRNEYISHAFKITKDGLDVLRRAKGASKHVRVPKRVYWEMFATNINDRVYVRTRRAYTLYLLMRSNTALNTVQLQVKLKALGFEELEETIENDVKGLINSGIFINVTNKGYHFKDTIKPFEIPEFGVTEPLVKGEMEKKKSDLRHKLKHVPHEYIELIEIAQDSKQNRLFEFKVVEFLKEVYDYNGKHLGGSRKPDGALYTNGLKTDYGIILDTKAYKDGYSLPISQADEMQRYVDENNNRNAIINPNEWWKVYPNSILDFKFLFVSGFFKGDYKKQLARVSNLTKRKGAVLSVEQLLLGGEKIKDGSLTLEDVGDKFNNDEIIF